European Patent Specification EP 4 095 247 B1, published June 10, 2026. Title: System for screening of agent for treating coronavirus disease. Applicant: Korea Institute of Oriental Medicine. The sequence listing filed with the application follows.

SEQUENCE LISTING (8 sequences)

SEQ ID NO: 1 - DNA, 2798 bp, Artificial Sequence
  recombinant MERS-CoV nsp12
tctaaagattccaattttttaaacgagtccggggttctattgtaaatgcccgaatagaaccctgttcaagtggtttgtccactgatgtcgtctttagggcatttgacatctgcaactataaggctaaggttgctggtattggaaaatactacaagactaatacttgtaggtttgtagaattagatgaccaagggcatcatttagactcctattttgtcgttaagaggcatactatggagaattatgaactagagaagcactgttacgatttgttacgtgactgtgatgctgtagctccccatgatttcttcatctttgatgtagacaaagttaaaacacctcatattgtacgtcagcgtttaactgagtacactatgatggatcttgtatatgccctgaggcactttgatcaaaatagcgaagtgcttaaggctatcttagtgaagtatggttgctgtgatgttacctactttgaaaataaactctggtttgattttgttgaaaatcccagtgttattggtgtttatcataaacttggagaacgtgtacgccaagctatcttaaacactgttaaattttgtgaccacatggtcaaggctggtttagtcggtgtgctcacactagacaaccaggaccttaatggcaagtggtatgattttggtgacttcgtaatcactcaacctggttcaggagtagctatagttgatagctactattcttatttgatgcctgtgctctcaatgaccgattgtctggccgctgagacacatagggattgtgattttaataaaccactcattgagtggccacttactgagtatgattttactgattataaggtacaactctttgagaagtactttaaatattgggatcagacgtatcacgcaaattgcgttaattgtactgatgaccgttgtgtgttacattgtgctaatttcaatgtattgtttgctatgaccatgcctaagacttgtttcggacccatagtccgaaagatctttgttgatggcgtgccatttgtagtatcttgtggttatcactacaaagaattaggtttagtcatgaatatggatgttagtctccatagacataggctctctcttaaggagttgatgatgtatgccgctgatccagccatgcacattgcctcctctaacgcttttcttgatttgaggacatcatgttttagtgtcgctgcacttacaactggtttgacttttcaaactgtgcggcctggcaattttaaccaagacttctatgatttcgtggtatctaaaggtttctttaaggagggctcttcagttacgctcaaacattttttctttgctcaagatggtaatgctgctattacagattataattactattcttataatctgcctactatgtgtgacatcaaacaaatgttgttctgcatggaagttgtaaacaagtacttcgaaatctatgacggtggttgtcttaatgcttctgaagtggttgttaataatttagacaagagtgctggccatccttttaataagtttggcaaagctcgtgtctattatgagagcatgtcttaccaggagcaagatgaactctttgccatgacaaagcgtaacgtcattcctaccatgactcaaatgaatctaaaatatgctattagtgctaagaatagagctcgcactgttgcaggcgtgtccatacttagcacaatgactaatcgccagtaccatcagaaaatgcttaagtccatggctgcaactcgtggagcgacttgcgtcattggtactacaaagttctatggtggctgggatttcatgcttaaaacattgtacaaagatgttgataatccgcatcttatgggttgggattaccctaagtgtgatagagctatgcctaatatgtgtagaatcttcgcttcactcatattagctcgtaaacatggcacttgttgtactacaagggacagattttatcgcttggcaaatgagtgtgctcaggtgctaagcgaatatgttctatgtggtggtggttactacgtcaaacctggaggtaccagtagcggagatgccaccactgcatatgccaatagtgtctttaacattttgcaggcgacaactgctaatgtcagtgcacttatgggtgctaatggcaacaagattgttgacaaagaagttaaagacatgcagtttgatttgtatgtcaatgtttacaggagcactagcccagaccccaaatttgttgataaatactatgcttttcttaataagcacttttctatgatgatactgtctgatgacggtgtcgtttgctataatagtgattatgcagctaagggttacattgctggaatacagaattttaaggaaacgctgtattatcagaacaatgtctttatgtctgaagctaaatgctgggtggaaaccgatctgaagaaagggccacatgaattctgttcacagcatacgctttatattaaggatggcgacgatggttacttccttccttatccagacccttcaagaattttgtctgccggttgctttgtagatgatatcgttaagactgacggtacactcatggtagagcggtttgtgtctttggctatagatgcttaccctctcacaaagcatgaagatatagaataccagaatgtattctgggtctacttacagtatatagaaaaactgtataaagaccttacaggacacatgcttgacagttattctgtcatgctatgtggtgataattctgctaagttttgggaagaggcattctacagagatctctatagttcgcctaccactttgcag

SEQ ID NO: 2 - DNA, 2796 bp, Artificial Sequence
  recombinant SARS-CoV nsp12
tcagctgatgcacaatcgtttttaaacgggtttgcggtgtaagtgcagcccgtcttacaccgtgcggcacaggcactagtactgatgtcgtatacagggcttttgacatctacaatgataaagtagctggttttgctaaattcctaaaaactaattgttgtcgcttccaagaaaaggacgaagatgacaatttaattgattcttactttgtagttaagagacacactttctctaactaccaacatgaagaaacaatttataatttacttaaggattgtccagctgttgctaaacatgacttctttaagtttagaatagacggtgacatggtaccacatatatcacgtcaacgtcttactaaatacacaatggcagacctcgtctatgctttaaggcattttgatgaaggtaattgtgacacattaaaagaaatacttgtcacatacaattgttgtgatgatgattatttcaataaaaaggactggtatgattttgtagaaaacccagatatattacgcgtatacgccaacttaggtgaacgtgtacgccaagctttgttaaaaacagtacaattctgtgatgccatgcgaaatgctggtattgttggtgtactgacattagataatcaagatctcaatggtaactggtatgatttcggtgatttcatacaaaccacgccaggtagtggagttcctgttgtagattcttattattcattgttaatgcctatattaaccttgaccagggctttaactgcagagtcacatgttgacactgacttaacaaagccttacattaagtgggatttgttaaaatatgacttcacggaagagaggttaaaactctttgaccgttattttaaatattgggatcagacataccacccaaattgtgttaactgtttggatgacagatgcattctgcattgtgcaaactttaatgttttattctctacagtgttcccacctacaagttttggaccactagtgagaaaaatatttgttgatggtgttccatttgtagtttcaactggataccacttcagagagctaggtgttgtacataatcaggatgtaaacttacatagctctagacttagttttaaggaattacttgtgtatgctgctgaccctgctatgcacgctgcttctggtaatctattactagataaacgcactacgtgcttttcagtagctgcacttactaacaatgttgcttttcaaactgtcaaacccggtaattttaacaaagacttctatgactttgctgtgtctaagggtttctttaaggaaggaagttctgttgaattaaaacacttcttctttgctcaggatggtaatgctgctatcagcgattatgactactatcgttataatctaccaacaatgtgtgatatcagacaactactatttgtagttgaagttgttgataagtactttgattgttacgatggtggctgtattaatgctaaccaagtcatcgtcaacaacctagacaaatcagctggttttccatttaataaatggggtaaggctagactttattatgattcaatgagttatgaggatcaagatgcacttttcgcatatacaaaacgtaatgtcatccctactataactcaaatgaatcttaagtatgccattagtgcaaagaatagagctcgcaccgtagctggtgtctctatctgtagtactatgaccaatagacagtttcatcaaaaattattgaaatcaatagccgccactagaggagctactgtagtaattggaacaagcaaattctatggtggttggcacaacatgttaaaaactgtttatagtgatgtagaaaaccctcaccttatgggttgggattatcctaaatgtgatagagccatgcctaacatgcttagaattatggcctcacttgttcttgctcgcaaacatacaacgtgttgtagcttgtcacaccgtttctatagattagctaatgagtgtgctcaagtattgagtgaaatggtcatgtgtggcggttcactatatgttaaaccaggtggaacctcatcaggagatgccacaactgcttatgctaatagtgtttttaacatttgtcaagctgtcacggccaatgttaatgcacttttatctactgatggtaacaaaattgccgataagtatgtccgcaatttacaacacagactttatgagtgtctctatagaaatagagatgttgacacagactttgtgaatgagttttacgcatatttgcgtaaacatttctcaatgatgatactctctgacgatgctgttgtgtgtttcaatagcacttatgcatctcaaggtctagtggctagcataaagaactttaagtcagttctttattatcaaaacaatgtttttatgtctgaagcaaaatgttggactgagactgaccttactaaaggacctcatgaattttgctctcaacatacaatgctagttaaacagggtgatgattatgtgtaccttccttacccagatccatcaagaatcctaggggccggctgttttgtagatgatatcgtaaaaacagatggtacacttatgattgaacggttcgtgtctttagctatagatgcttacccacttactaaacatcctaatcaggagtatgctgatgtctttcatttgtacttacaatacataagaaagctacatgatgagttaacaggacacatgttagacatgtattctgttatgcttactaatgataacacttcaaggtattgggaacctgagttttatgaggctatgtacacaccgcatacagtcttacagg

SEQ ID NO: 3 - DNA, 249 bp, Artificial Sequence
  recombinant MERS-CoV nsp7
tctaaacttacagatcttaaatgcacatctgtggttctcctctctgtgctccaacagttacacttagaggctaatagtagggcctgggctttctgtgttaaatgccataatgacatattggcagcaacagaccccagtgaggctttcgagaaattcgtaagtctctttgccactttaatgactttttctggtaatgtagatcttgatgcgttagctagtgatatttttgacactcctagcgtacttcaa

SEQ ID NO: 4 - DNA, 249 bp, Artificial Sequence
  recombinant SARS-CoV nsp7
tctaaaatgtcagatgtaaagtgcacatcagtagtcttactctcagttttgcaacaactcagagtagaatcatcatctaaattgtgggctcaatgtgtccagttacacaatgacattctcttagctaaagatactactgaagcctttgaaaaaatggtttcactactttctgttttgctttccatgcagggtgctgtagacataaacaagctttgtgaagaaatgctggacaacagggcaaccttacaa

SEQ ID NO: 5 - DNA, 597 bp, Artificial Sequence
  recombinant MERS-CoV nsp8
gctactctttctgagttttcacacttagctacctttgctgagttggaagctgcgcagaaagcctatcaggaagctatggactctggtgacacctcaccacaagttcttaaggctttgcagaaggctgttaatatagctaaaaacgcctatgagaaggataaggcagtggcccgtaagttagaacgtatggctgatcaggctatgacttctatgtataagcaagcacgtgctgaagacaagaaagcaaaaattgtcagtgctatgcaaactatgttgtttggtatgattaagaagctcgacaacgatgttcttaatggtatcatttctaacgctaggaatggttgtatacctcttagtgtcattccactgtgtgcttcaaataaacttcgcgttgtaattcctgacttcaccgtctggaatcaggtagtcacatatccctcgcttaactacgctggggctttgtgggacattacagttataaacaatgtggacaatgaaattgttaagtcttcagatgttgtagacagcaatgaaaatttaacatggccacttgttttagaatgcactagggcatccacttctgccgttaagttgcaa

SEQ ID NO: 6 - DNA, 594 bp, Artificial Sequence
  recombinant SARS-CoV nsp8
gctatagcctcagagtttagttcccttccatcatatgcagcttttgctactgctcaagaagcttatgagcaggctgttgctaatggtgattctgaagttgttcttaaaaagttgaagaagtctttgaatgtggctaaatctgaatttgaccgtgatgcagccatgcaacgtaagttggaaaagatggctgatcaagctatgacccaaatgtataaacaggctagatctgaggacaagagggcaaaagttactagtgctatgcagacaatgcttttcactatgcttagaaagttggataatgatgcactcaacaacattatcaacaatgcaagagatggttgtgttcccttgaacataatacctcttacaacagcagccaaactaatggttgtcataccagactataacacatataaaaatacgtgtgatggtacaacatttacttatgcatcagcattgtgggaaatccaacaggttgtagatgcagatagtaaaattgttcaacttagtgaaattagtatggacaattcacctaatttagcatggcctcttattgtaacagctttaagggccaattctgctgtcaaattacag

SEQ ID NO: 7 - DNA, 1653 bp, Artificial Sequence
  recombinant FLuc
atggaagacgccaaaaacataaagaaaggcccggcgccattctatccgctggaagatggaaccgctggagagcaactgcataaggctatgaagagatacgccctggttcctggaacaattgcttttacagatgcacatatcgaggtggacatcacttacgctgagtacttcgaaatgtccgttcggttggcagaagctatgaaacgatatgggctgaatacaaatcacagaatcgtcgtatgcagtgaaaactctcttcaattctttatgccggtgttgggcgcgttatttatcggagttgcagttgcgcccgcgaacgacatttataatgaacgtgaattgctcaacagtatgggcatttcgcagcctaccgtggtgttcgtttccaaaaaggggttgcaaaaaattttgaacgtgcaaaaaaagctcccaatcatccaaaaaattattatcatggattctaaaacggattaccagggatttcagtcgatgtacacgttcgtcacatctcatctacctcccggttttaatgaatacgattttgtgccagagtccttcgatagggacaagacaattgcactgatcatgaactcctctggatctactggtctgcctaaaggtgtcgctctgcctcatagaactgcctgcgtgagattctcgcatgccagagatcctatttttggcaatcaaatcattccggatactgcgattttaagtgttgttccattccatcacggttttggaatgtttactacactcggatatttgatatgtggatttcgagtcgtcttaatgtatagatttgaagaagagctgtttctgaggagccttcaggattacaagattcaaagtgcgctgctggtgccaaccctattctccttcttcgccaaaagcactctgattgacaaatacgatttatctaatttacacgaaattgcttctggtggcgctcccctctctaaggaagtcggggaagcggttgccaagaggttccatctgccaggtatcaggcaaggatatgggctcactgagactacatcagctattctgattacacccgagggggatgataaaccgggcgcggtcggtaaagttgttccattttttgaagcgaaggttgtggatctggataccgggaaaacgctgggcgttaatcaaagaggcgaactgtgtgtgagaggtcctatgattatgtccggttatgtaaacaatccggaagcgaccaacgccttgattgacaaggatggatggctacattctggagacatagcttactgggacgaagacgaacacttcttcatcgttgaccgcctgaagtctctgattaagtacaaaggctatcaggtggctcccgctgaattggaatccatcttgctccaacaccccaacatcttcgacgcaggtgtcgcaggtcttcccgacgatgacgccggtgaacttcccgccgccgttgttgttttggagcacggaaagacgatgacggaaaaagagatcgtggattacgtcgccagtcaagtaacaaccgcgaaaaagttgcgcggaggagttgtgtttgtggacgaagtaccgaaaggtcttaccggaaaactcgacgcaagaaaaatcagagagatcctcataaaggccaagaagggcggaaagatcgccgtgtaa

SEQ ID NO: 8 - DNA, 516 bp, Artificial Sequence
  recombinant NLuc
atggtcttcacactcgaagatttcgttggggactggcgacagacagccggctacaacctggaccaagtccttgaacagggaggtgtgtccagtttgtttcagaatctcggggtgtccgtaactccgatccaaaggattgtcctgagcggtgaaaatgggctgaagatcgacatccatgtcatcatcccgtatgaaggtctgagcggcgaccaaatgggccagatcgaaaaaatttttaaggtggtgtaccctgtggatgatcatcactttaaggtgatcctgcactatggcacactggtaatcgacggggttacgccgaacatgatcgactatttcggacggccgtatgaaggcatcgccgtgttcgacggcaaaaagatcactgtaacagggaccctgtggaacggcaacaaaattatcgacgagcgcctgatcaaccccgacggctccctgctgttccgagtaaccatcaacggagtgaccggctggcggctgtgcgaacgcattctggcgtaa